European Patent Specification EP 3 414 266 B1, published July 16, 2025. Title: Broadly Neutralizing Antibodies against HIV-1 and Use thereof. Applicant: National Center for AIDS/STD Control and Prevention, Chinese Center for Disease Control and Prevention The Scripps Research Institute. The sequence listing filed with the application follows.

SEQUENCE LISTING (10 sequences)

SEQ ID NO: 1 - DNA, 360 bp, Homo sapiens
caggtgcagctggtggagtctgggactcaatttaggaggcctggggcctcagtgagactctcctgcgaggcttctggatacaccttcatctcctcctttatacattggataaggcagggccctggccaagggcttgagtggatggggtggatgaaccctagacatggcgccgttaattacccgcggaggtttcagggtaaggtgaccatgaccagggacacgtccatcgacacagcctacatggagctgcgtgacctgagatctgacgacacggccatgtatttctgtgtgacatctcggactaaagactatgactgggactttgtctggggccaggggaccctggtcgtcgtctcctca

SEQ ID NO: 2 - protein, 120 aa, Homo sapiens
QVQLVESGTQFRRPGASVRLSCEASGYTFISSFIHWIRQGPGQGLEWMGWMNPRHGAVNYPRRFQGKVTMTRDTSIDTAYMELRDLRSDDTAMYFCVTSRTKDYDWDFVWGQGTLVVVSS

SEQ ID NO: 3 - DNA, 360 bp, Homo sapiens
cagaaacaactggtgcagtctgggactcaatttaagaggcctggggcctcagtgagactctcctgcgaggcttctggatacaccttcatctcctccttcatacattggataaggcagggccctggccaaggacttgagtggatggggtggatgaatcctagacatggcggcgtaaattaccctcggaggtttcagggtaaggtcaccatgaccagggacacgtccatcgacacagcctacatggagctgcgtgacctgagatctgacgacacggccatgtatttctgtgtgacctcccggactaaagactatgactgggactttgtctggggccaggggaccctggtcgtcgtctcctca

SEQ ID NO: 4 - protein, 120 aa, Homo sapiens
QKQLVQSGTQFKRPGASVRLSCEASGYTFISSFIHWIRQGPGQGLEWMGWMNPRHGGVNYPRRFQGKVTMTRDTSIDTAYMELRDLRSDDTAMYFCVTSRTKDYDWDFVWGQGTLVVVSS

SEQ ID NO: 5 - DNA, 360 bp, Homo sapiens
cagagacaactggtgcagtctgggactcagtttaagaggcctggggcctcagtgagactctcctgcgaggcttctggatacaccttcatctcatcctttatacactggatacgacaggcccctggccaaggccttgagtggatggggtggatgaaccctagacatggcgccgtgaattaccctcggaggtttcagggtaaggtcaccatgtccagggacacgtctatcgacacagcctacatggagctgcgtgacctgagagctgacgacacggccacttatttctgtgtgacctcccggactaatgactatgactgggactttgtctggggccaggggaccctggtcgtcgtctcctca

SEQ ID NO: 6 - protein, 120 aa, Homo sapiens
QRQLVQSGTQFKRPGASVRLSCEASGYTFISSFIHWIRQAPGQGLEWMGWMNPRHGAVNYPRRFQGKVTMSRDTSIDTAYMELRDLRADDTATYFCVTSRTNDYDWDFVWGQGTLVVVSS

SEQ ID NO: 7 - DNA, 309 bp, Homo sapiens
gacatccagatgacccagtctccagtcaccctgtctgcgtctataggagacagagtcaccatcacttgtcgggccagtcagaggatagataactgggtggcctggtatcagcagaaaccagggagagcccctaaactcctcatctataaggcctctattttagagacaggggtcccatctcgattcagcggcagtgggtctgggacagaattcactctctccatcaacagcctgcagcctgatgatgtcgcaacttattactgccaacaatttgaggagttcggccgagggaccaagattgacatcaaa

SEQ ID NO: 8 - protein, 103 aa, Homo sapiens
DIQMTQSPVTLSASIGDRVTITCRASQRIDNWVAWYQQKPGRAPKLLIYKASILETGVPSRFSGSGSGTEFTLSINSLQPDDVATYYCQQFEEFGRGTKIDIK

SEQ ID NO: 9 - DNA, 315 bp, Homo sapiens
gaaattgtgttgacacagtctccaggcaccctgtctttgtctccaggggaaacagccatcatctcttgtcggaccagtcagtatggttccttagcctggtatcaacagaggcccggccaggcccccaggctcgtcatctattcgggctctactcgggccgctggcatcccagacaggttcagcggcagtcggtgggggccagactacaatctcaccatcagcaacctggagtcgggagattttggtgtttattattgccagcagtatgaattttttggccaggggaccaaggtccaggtcgacattaaacgtacg

SEQ ID NO: 10 - protein, 105 aa, Homo sapiens
EIVLTQSPGTLSLSPGETAIISCRTSQYGSLAWYQQRPGQAPRLVIYSGSTRAAGIPDRFSGSRWGPDYNLTISNLESGDFGVYYCQQYEFFGQGTKVQVDIKRT